European Patent Application EP 4 628 528 A1, published October 8, 2025. Title: ALGINATE HYDROGEL PARTICLES FOR CELL CULTURE APPLICATIONS. Applicant: Nutrition Biosciences USA. Application US. The sequence listing filed with the application follows.

SEQUENCE LISTING (6 sequences)

SEQ ID NO: 1 - protein, 7 aa, synthetic construct
GRGDSPK

SEQ ID NO: 2 - protein, 15 aa, synthetic construct
KGGNGEPRGDTYRAY

SEQ ID NO: 3 - protein, 12 aa, synthetic construct
NGEPRGDTYRAY

SEQ ID NO: 4 - protein, 12 aa, synthetic construct
AVTGRGDSPASS

SEQ ID NO: 5 - protein, 12 aa, synthetic construct
PQVTRGDVFTMP

SEQ ID NO: 6 - protein, 6 aa, synthetic construct
GRGDSP